European Patent Specification EP 3 603 648 B1, published September 17, 2025. Title: Complex of nucleic acid medicine and multibranched lipid. Applicant: SHIONOGI & CO., LTD. The sequence listing filed with the application follows.

SEQUENCE LISTING (15 sequences)

SEQ ID NO: 1 - RNA, 19 nt, Artificial sequence
  Antisense oligonucleotide of Hprt1 siRNA
uuaaaguugagagaucauc

SEQ ID NO: 2 - RNA, 19 nt, Artificial sequence
  Sense oligonucleotide of Hprt1 siRNA
gaugaucucucaacuuuaa

SEQ ID NO: 3 - RNA, 21 nt, Artificial sequence
  Antisense oligonucleotide of Luc siRNA
guaggaguagugaaaggccag

SEQ ID NO: 4 - RNA, 21 nt, Artificial sequence
  Sense oligonucleotide of Luc siRNA
ggccuuucacuacuccuacga

SEQ ID NO: 5 - DNA, 21 bp, Artificial sequence
  Primer
ctaccctctggtagattgtcg

SEQ ID NO: 6 - DNA, 22 bp, Artificial sequence
  Primer
tcgagagcttcagactcgtcta

SEQ ID NO: 7 - DNA, 20 bp, Artificial sequence
  Primer
gcaccgtcaaggctgagaac

SEQ ID NO: 8 - DNA, 19 bp, Artificial sequence
  Primer
tggtgaagacgccagtgga

SEQ ID NO: 9 - DNA, 25 bp, Artificial sequence
  Primer
ttgttgttggatatgcccttgacta

SEQ ID NO: 10 - DNA, 21 bp, Artificial sequence
  Primer
aggcagatggccacaggacta

SEQ ID NO: 11 - DNA, 20 bp, Artificial sequence
  Primer
tgtgtccgtcgtggatctga

SEQ ID NO: 12 - DNA, 21 bp, Artificial sequence
  Primer
ttgctgttgaagtcgcaggag

SEQ ID NO: 13 - RNA, 16 nt, Artificial sequence
  Sense oligonucleotide of Hprt1 siRNA
gaucucucaacuuuaa

SEQ ID NO: 14 - protein, 5 aa, Artificial sequence
  Amino acid linker
WCAAK

SEQ ID NO: 15 - protein, 5 aa, Artificial sequence
  Amino acid linker
WCKVK